European Patent Specification EP 3 638 302 B1, published March 13, 2024. Title: POXVIRUS VECTORS ENCODING HIV ANTIGENS, AND METHODS OF USE THEREOF. Applicant: Janssen Vaccines & Prevention B.V. Bavarian Nordic A/S. The sequence listing filed with the application follows.

SEQUENCE LISTING (46 sequences)

SEQ ID NO: 1 - protein, 500 aa, Artificial Sequence
  mos1Gag mosaic antigen sequence
MGARASVLSGGELDRWEKIRLRPGGKKKYRLKHIVWASRELERFAVNPGLLETSEGCRQILGQLQPSLQTGSEELRSLYNTVATLYCVHQRIEIKDTKEALEKIEEEQNKSKKKAQQAAADTGNSSQVSQNYPIVQNIQGQMVHQAISPRTLNAWVKVVEEKAFSPEVIPMFSALSEGATPQDLNTMLNTVGGHQAAMQMLKETINEEAAEWDRVHPVHAGPIAPGQMREPRGSDIAGTTSTLQEQIGWMTNNPPIPVGEIYKRWIILGLNKIVRMYSPVSILDIRQGPKEPFRDYVDRFYKTLRAEQASQDVKNWMTETLLVQNANPDCKTILKALGPAATLEEMMTACQGVGGPGHKARVLAEAMSQVTNSATIMMQRGNFRNQRKTVKCFNCGKEGHIAKNCRAPRKKGCWKCGKEGHQMKDCTERQANFLGKIWPSNKGRPGNFLQNRPEPTAPPEESFRFGEETTTPSQKQEPIDKEMYPLASLKSLFGNDPSSQ

SEQ ID NO: 2 - protein, 491 aa, Artificial Sequence
  mos2Gag mosaic antigen sequence
MGARASILRGGKLDKWEKIRLRPGGKKHYMLKHLVWASRELERFALNPGLLETSEGCKQIIKQLQPALQTGTEELRSLFNTVATLYCVHAEIEVRDTKEALDKIEEEQNKSQQKTQQAKEADGKVSQNYPIVQNLQGQMVHQPISPRTLNAWVKVIEEKAFSPEVIPMFTALSEGATPQDLNTMLNTVGGHQAAMQMLKDTINEEAAEWDRLHPVHAGPVAPGQMREPRGSDIAGTTSNLQEQIAWMTSNPPIPVGDIYKRWIILGLNKIVRMYSPTSILDIKQGPKEPFRDYVDRFFKTLRAEQATQDVKNWMTDTLLVQNANPDCKTILRALGPGATLEEMMTACQGVGGPSHKARVLAEAMSQTNSTILMQRSNFKGSKRIVKCFNCGKEGHIARNCRAPRKKGCWKCGKEGHQMKDCTERQANFLGKIWPSHKGRPGNFLQSRPEPTAPPAESFRFEETTPAPKQEPKDREPLTSLRSLFGSDPLSQ

SEQ ID NO: 3 - protein, 850 aa, Artificial Sequence
  mos1Pol mosaic antigen sequence
MAPISPIETVPVKLKPGMDGPRVKQWPLTEEKIKALTAICEEMEKEGKITKIGPENPYNTPVFAIKKKDSTKWRKLVDFRELNKRTQDFWEVQLGIPHPAGLKKKKSVTVLAVGDAYFSVPLDEGFRKYTAFTIPSTNNETPGIRYQYNVLPQGWKGSPAIFQCSMTRILEPFRAKNPEIVIYQYMAALYVGSDLEIGQHRAKIEELREHLLKWGFTTPDKKHQKEPPFLWMGYELHPDKWTVQPIQLPEKDSWTVNDIQKLVGKLNWASQIYPGIKVRQLCKLLRGAKALTDIVPLTEEAELELAENREILKEPVHGVYYDPSKDLIAEIQKQGHDQWTYQIYQEPFKNLKTGKYAKMRTAHTNDVKQLTEAVQKIAMESIVIWGKTPKFRLPIQKETWETWWTDYWQATWIPEWEFVNTPPLVKLWYQLEKDPIAGVETFYVAGAANRETKLGKAGYVTDRGRQKIVSLTETTNQKTALQAIYLALQDSGSEVNIVTASQYALGIIQAQPDKSESELVNQIIEQLIKKERVYLSWVPAHKGIGGNEQVDKLVSSGIRKVLFLDGIDKAQEEHEKYHSNWRAMASDFNLPPVVAKEIVASCDQCQLKGEAMHGQVDCSPGIWQLACTHLEGKIILVAVHVASGYIEAEVIPAETGQETAYFILKLAGRWPVKVIHTANGSNFTSAAVKAACWWAGIQQEFGIPYNPQSQGVVASMNKELKKIIGQVRDQAEHLKTAVQMAVFIHNFKRKGGIGGYSAGERIIDIIATDIQTKELQKQIIKIQNFRVYYRDSRDPIWKGPAKLLWKGEGAVVIQDNSDIKVVPRRKVKIIKDYGKQMAGADCVAGRQDED

SEQ ID NO: 4 - protein, 850 aa, Artificial Sequence
  mos2Pol mosaic antigen sequence
MAPISPIETVPVKLKPGMDGPKVKQWPLTEEKIKALVEICTEMEKEGKISKIGPENPYNTPIFAIKKKDSTKWRKLVDFRELNKRTQDFWEVQLGIPHPAGLKKKKSVTVLAVGDAYFSVPLDEDFRKYTAFTIPSINNETPGIRYQYNVLPQGWKGSPAIFQSSMTKILEPFRKQNPDIVIYQYMAALYVGSDLEIGQHRTKIEELRQHLLRWGFTTPDKKHQKEPPFLWMGYELHPDKWTVQPIVLPEKDSWTVNDIQKLVGKLNWASQIYAGIKVKQLCKLLRGTKALTEVVPLTEEAELELAENREILKEPVHGVYYDPSKDLIAEIQKQGQGQWTYQIYQEPFKNLKTGKYARMRGAHTNDVKQLTEAVQKIATESIVIWGKTPKFKLPIQKETWEAWWTEYWQATWIPEWEFVNTPPLVKLWYQLEKEPIVGAETFYVAGAANRETKLGKAGYVTDRGRQKVVSLTDTTNQKTALQAIHLALQDSGLEVNIVTASQYALGIIQAQPDKSESELVSQIIEQLIKKEKVYLAWVPAHKGIGGNEQVDKLVSRGIRKVLFLDGIDKAQEEHEKYHSNWRAMASEFNLPPIVAKEIVASCDKCQLKGEAIHGQVDCSPGIWQLACTHLEGKVILVAVHVASGYIEAEVIPAETGQETAYFLLKLAGRWPVKTIHTANGSNFTSATVKAACWWAGIKQEFGIPYNPQSQGVVASINKELKKIIGQVRDQAEHLKTAVQMAVFIHNFKRKGGIGEYSAGERIVDIIASDIQTKELQKQITKIQNFRVYYRDSRDPLWKGPAKLLWKGEGAVVIQDNSDIKVVPRRKAKIIRDYGKQMAGDDCVASRQDED

SEQ ID NO: 5 - protein, 685 aa, Artificial Sequence
  mos1Env mosaic antigen sequence
MRVTGIRKNYQHLWRWGTMLLGILMICSAAGKLWVTVYYGVPVWKEATTTLFCASDAKAYDTEVHNVWATHACVPTDPNPQEVVLENVTENFNMWKNNMVEQMHEDIISLWDQSLKPCVKLTPLCVTLNCTDDVRNVTNNATNTNSSWGEPMEKGEIKNCSFNITTSIRNKVQKQYALFYKLDVVPIDNDSNNTNYRLISCNTSVITQACPKVSFEPIPIHYCAPAGFAILKCNDKKFNGTGPCTNVSTVQCTHGIRPVVSTQLLLNGSLAEEEVVIRSENFTNNAKTIMVQLNVSVEINCTRPNNNTRKSIHIGPGRAFYTAGDIIGDIRQAHCNISRANWNNTLRQIVEKLGKQFGNNKTIVFNHSSGGDPEIVMHSFNCGGEFFYCNSTKLFNSTWTWNNSTWNNTKRSNDTEEHITLPCRIKQIINMWQEVGKAMYAPPIRGQIRCSSNITGLLLTRDGGNDTSGTEIFRPGGGDMRDNWRSELYKYKVVKIEPLGVAPTKAKRRVVQSEKSAVGIGAVFLGFLGAAGSTMGAASMTLTVQARLLLSGIVQQQNNLLRAIEAQQHLLQLTVWGIKQLQARVLAVERYLKDQQLLGIWGCSGKLICTTTVPWNASWSNKSLDKIWNNMTWMEWEREINNYTSLIYTLIEESQNQQEKNEQELLELDKWASLWNWFDISNWLW

SEQ ID NO: 6 - protein, 684 aa, Artificial Sequence
  mos2Env mosaic antigen sequence
MRVRGIQRNWPQWWIWGILGFWMIIICRVMGNLWVTVYYGVPVWKEAKTTLFCASDAKAYEKEVHNVWATHACVPTDPNPQEMVLENVTENFNMWKNDMVDQMHEDIIRLWDQSLKPCVKLTPLCVTLECRNVRNVSSNGTYNIIHNETYKEMKNCSFNATTVVEDRKQKVHALFYRLDIVPLDENNSSEKSSENSSEYYRLINCNTSAITQACPKVSFDPIPIHYCAPAGYAILKCNNKTFNGTGPCNNVSTVQCTHGIKPVVSTQLLLNGSLAEEEIIIRSENLTNNAKTIIVHLNETVNITCTRPNNNTRKSIRIGPGQTFYATGDIIGDIRQAHCNLSRDGWNKTLQGVKKKLAEHFPNKTINFTSSSGGDLEITTHSFNCRGEFFYCNTSGLFNGTYMPNGTNSNSSSNITLPCRIKQIINMWQEVGRAMYAPPIAGNITCRSNITGLLLTRDGGSNNGVPNDTETFRPGGGDMRNNWRSELYKYKVVEVKPLGVAPTEAKRRVVESEKSAVGIGAVFLGILGAAGSTMGAASITLTVQARQLLSGIVQQQSNLLRAIEAQQHMLQLTVWGIKQLQTRVLAIERYLQDQQLLGLWGCSGKLICTTAVPWNTSWSNKSQTDIWDNMTWMQWDKEIGNYTGEIYRLLEESQNQQEKNEKDLLALDSWKNLWNWFDITNWLW

SEQ ID NO: 7 - protein, 708 aa, Artificial Sequence
  stabilized clade C gp140 trimer: C97ZA012-gp140-foldon with cleavage mutations
MRVRGIQRNCQHLWRWGTLILGMLMICSAAENLWVGNMWVTVYYGVPVWTDAKTTLFCASDTKAYDREVHNVWATHACVPTDPNPQEIVLENVTENFNMWKNDMVDQMHEDIISLWDQSLKPCVKLTPLCVTLHCTNATFKNNVTNDMNKEIRNCSFNTTTEIRDKKQQGYALFYRPDIVLLKENRNNSNNSEYILINCNASTITQACPKVNFDPIPIHYCAPAGYAILKCNNKTFSGKGPCNNVSTVQCTHGIKPVVSTQLLLNGSLAEKEIIIRSENLTDNVKTIIVHLNKSVEIVCTRPNNNTRKSMRIGPGQTFYATGDIIGDIRQAYCNISGSKWNETLKRVKEKLQENYNNNKTIKFAPSSGGDLEITTHSFNCRGEFFYCNTTRLFNNNATEDETITLPCRIKQIINMWQGVGRAMYAPPIAGNITCKSNITGLLLVRDGGEDNKTEEIFRPGGGNMKDNWRSELYKYKVIELKPLGIAPTGAKERVVEREERAVGIGAVFLGFLGAAGSTMGAASLTLTVQARQLLSSIVQQQSNLLRAIEAQQHMLQLTVWGIKQLQTRVLAIERYLKDQQLLGIWGCSGKLICTTNVPWNSSWSNKSQTDIWNNMTWMEWDREISNYTDTIYRLLEDSQTQQEKNEKDLLALDSWKNLWSWFDISNWLWYIKSRIEGRGSGGYIPEAPRDGQAYVRKDGEWVLLSTFL

SEQ ID NO: 8 - protein, 625 aa, Artificial Sequence
  C4 fragment: gp120-truncated gp41 without signal peptide and transmembrane domain
MGNLWVTVYYGVPVWKDAKTTLFCASDAKAYEKEVHNVWATHACVPTDPNPQEIVLGNVTENFNMWKNDMVDQMHEDIISLWDASLEPCVKLTPLCVTLNCRNVRNVSSNGTYNIIHNETYKEMKNCSFNATTVVEDRKQKVHALFYRLDIVPLDENNSSEKSSENSSEYYRLINCNTSAITQACPKVSFDPIPIHYCAPAGYAILKCNNKTFNGTGPCNNVSTVQCTHGIKPVVSTQLLLNGSLAEEEIIIRSENLTNNAKTIIVHLNETVNITCTRPNNNTRKSIRIGPGQTFYATGDIIGDIRQAHCNLSRDGWNKTLQGVKKKLAEHFPNKTIKFAPHSGGDLEITTHTFNCRGEFFYCNTSNLFNESNIERNDSIITLPCRIKQIINMWQEVGRAIYAPPIAGNITCRSNITGLLLTRDGGSNNGVPNDTETFRPGGGDMRNNWRSELYKYKVVEVKPLGVAPTEAKRRVVEREKRAVGIGAVFLGILGAAGSTMGAASITLTVQARQLLSGIVQQQSNLLRAIEAQQHMLQLTVWGIKQLQTRVLAIERYLQDQQLLGLWGCSGKLICTTAVPWNTSWSNKSQTDIWDNMTWMQWDKEIGNYTGEIYRLLEESQNQQEK

SEQ ID NO: 9 - protein, 29 aa, Artificial Sequence
  signal sequence
MRVRGMLRNWQQWWIWSSLGFWMLMIYSV

SEQ ID NO: 10 - protein, 29 aa, Artificial Sequence
  signal sequence
MRVTGIRKNYQHLWRWGTMLLGILMICSA

SEQ ID NO: 11 - protein, 29 aa, Artificial Sequence
  signal sequence
MRVRGIQRNWPQWWIWGILGFWMIIICRV

SEQ ID NO: 12 - protein, 29 aa, Artificial Sequence
  signal sequence
MRVRGIQRNCQHLWRWGTLILGMLMICSA

SEQ ID NO: 13 - protein, 22 aa, Artificial Sequence
  transmembrane domain
IFIMIVGGLIGLRIIFAVLSIV

SEQ ID NO: 14 - protein, 7 aa, Artificial Sequence
  truncated cytoplasmic region
NRVRQGY

SEQ ID NO: 15 - protein, 32 aa, Artificial Sequence
  GCN4 trimerization domain
MKQIEDKIEEILSKIYHIENEIARIKKLIGEV

SEQ ID NO: 16 - protein, 30 aa, Artificial Sequence
  foldon trimerization domain
GSGGYIPEAPRDGQAYVRKDGEWVLLSTFL

SEQ ID NO: 17 - protein, 862 aa, Artificial Sequence
  C4 sequence
MRVRGMLRNWQQWWIWSSLGFWMLMIYSVMGNLWVTVYYGVPVWKDAKTTLFCASDAKAYEKEVHNVWATHACVPTDPNPQEIVLGNVTENFNMWKNDMVDQMHEDIISLWDASLEPCVKLTPLCVTLNCRNVRNVSSNGTYNIIHNETYKEMKNCSFNATTVVEDRKQKVHALFYRLDIVPLDENNSSEKSSENSSEYYRLINCNTSAITQACPKVSFDPIPIHYCAPAGYAILKCNNKTFNGTGPCNNVSTVQCTHGIKPVVSTQLLLNGSLAEEEIIIRSENLTNNAKTIIVHLNETVNITCTRPNNNTRKSIRIGPGQTFYATGDIIGDIRQAHCNLSRDGWNKTLQGVKKKLAEHFPNKTIKFAPHSGGDLEITTHTFNCRGEFFYCNTSNLFNESNIERNDSIITLPCRIKQIINMWQEVGRAIYAPPIAGNITCRSNITGLLLTRDGGSNNGVPNDTETFRPGGGDMRNNWRSELYKYKVVEVKPLGVAPTEAKRRVVEREKRAVGIGAVFLGILGAAGSTMGAASITLTVQARQLLSGIVQQQSNLLRAIEAQQHMLQLTVWGIKQLQTRVLAIERYLQDQQLLGLWGCSGKLICTTAVPWNTSWSNKSQTDIWDNMTWMQWDKEIGNYTGEIYRLLEESQNQQEKNEKDLLALDSWNNLWNWFSISKWLWYIKIFIMIVGGLIGLRIIFAVLSIVNRVRQGYSPLSLQTLTQNPGGLDRLGRIEEEGGEQDKDRSIRLVNGFFALFWDDLRSLCLFSYHRLRDFILIVARAVELLGRSSLRGLQRGWEILKYLGSLLQYWGLELKKSAINLLDTIAIAVAEGTDRIIELIQRICRAICNIPRRIRQGFEAALQ

SEQ ID NO: 18 - protein, 711 aa, Artificial Sequence
  C4D7 sequence
MRVRGMLRNWQQWWIWSSLGFWMLMIYSVMGNLWVTVYYGVPVWKDAKTTLFCASDAKAYEKEVHNVWATHACVPTDPNPQEIVLGNVTENFNMWKNDMVDQMHEDIISLWDASLEPCVKLTPLCVTLNCRNVRNVSSNGTYNIIHNETYKEMKNCSFNATTVVEDRKQKVHALFYRLDIVPLDENNSSEKSSENSSEYYRLINCNTSAITQACPKVSFDPIPIHYCAPAGYAILKCNNKTFNGTGPCNNVSTVQCTHGIKPVVSTQLLLNGSLAEEEIIIRSENLTNNAKTIIVHLNETVNITCTRPNNNTRKSIRIGPGQTFYATGDIIGDIRQAHCNLSRDGWNKTLQGVKKKLAEHFPNKTIKFAPHSGGDLEITTHTFNCRGEFFYCNTSNLFNESNIERNDSIITLPCRIKQIINMWQEVGRAIYAPPIAGNITCRSNITGLLLTRDGGSNNGVPNDTETFRPGGGDMRNNWRSELYKYKVVEVKPLGVAPTEAKRRVVEREKRAVGIGAVFLGILGAAGSTMGAASITLTVQARQLLSGIVQQQSNLLRAIEAQQHMLQLTVWGIKQLQTRVLAIERYLQDQQLLGLWGCSGKLICTTAVPWNTSWSNKSQTDIWDNMTWMQWDKEIGNYTGEIYRLLEESQNQQEKNEKDLLALDSWNNLWNWFSISKWLWYIKIFIMIVGGLIGLRIIFAVLSIVNRVRQGY

SEQ ID NO: 19 - protein, 704 aa, Artificial Sequence
  sC4 sequence
MRVRGMLRNWQQWWIWSSLGFWMLMIYSVMGNLWVTVYYGVPVWKDAKTTLFCASDAKAYEKEVHNVWATHACVPTDPNPQEIVLGNVTENFNMWKNDMVDQMHEDIISLWDASLEPCVKLTPLCVTLNCRNVRNVSSNGTYNIIHNETYKEMKNCSFNATTVVEDRKQKVHALFYRLDIVPLDENNSSEKSSENSSEYYRLINCNTSAITQACPKVSFDPIPIHYCAPAGYAILKCNNKTFNGTGPCNNVSTVQCTHGIKPVVSTQLLLNGSLAEEEIIIRSENLTNNAKTIIVHLNETVNITCTRPNNNTRKSIRIGPGQTFYATGDIIGDIRQAHCNLSRDGWNKTLQGVKKKLAEHFPNKTIKFAPHSGGDLEITTHTFNCRGEFFYCNTSNLFNESNIERNDSIITLPCRIKQIINMWQEVGRAIYAPPIAGNITCRSNITGLLLTRDGGSNNGVPNDTETFRPGGGDMRNNWRSELYKYKVVEVKPLGVAPTEAKRRVVEREERAVGIGAVFLGILGAAGSTMGAASITLTVQARQLLSGIVQQQSNLLRAIEAQQHMLQLTVWGIKQLQTRVLAIERYLQDQQLLGLWGCSGKLICTTAVPWNTSWSNKSQTDIWDNMTWMQWDKEIGNYTGEIYRLLEESQNQQEKMKQIEDKIEEILSKIYHIENEIARIKKLIGEVGSGAPTKAKRRVVQREKR

SEQ ID NO: 20 - DNA, 4050 bp, Artificial Sequence
  nucleotide sequence encoding mos1GagPol
atgggagccagagccagcgtgctgtccggaggggagctggaccgctgggagaagatcaggctgaggcctggagggaagaagaagtacaggctgaagcacatcgtgtgggccagcagagagctggaacggtttgccgtgaaccctggcctgctggaaaccagcgagggctgtaggcagattctgggacagctgcagcccagcctgcagacaggcagcgaggaactgcggagcctgtacaacaccgtggccaccctgtactgcgtgcaccagcggatcgagatcaaggacaccaaagaagccctggaaaagatcgaggaagagcagaacaagagcaagaagaaagcccagcaggctgccgctgacacaggcaacagcagccaggtgtcccagaactaccccatcgtgcagaacatccagggacagatggtgcaccaggccatcagccctcggaccctgaacgcctgggtgaaggtggtggaggaaaaggccttcagccctgaggtgatccccatgttctctgccctgagcgagggagccacaccccaggacctgaacaccatgctgaacaccgtgggagggcaccaggctgccatgcagatgctgaaagagacaatcaacgaggaagctgccgagtgggacagggtccacccagtgcacgctggacctatcgctcctggccagatgagagagcccagaggcagcgatattgctggcaccacctccacactgcaggaacagatcggctggatgaccaacaaccctcccatccctgtgggagagatctacaagcggtggatcattctgggactgaacaagatcgtgcggatgtacagccctgtgagcatcctggacatcaggcagggacccaaagagcccttcagggactacgtggaccggttctacaagaccctgagagccgagcaggccagccaggacgtgaagaactggatgaccgagacactgctggtgcagaacgccaaccctgactgcaagaccatcctgaaagccctgggacctgctgccaccctggaagagatgatgacagcctgccagggagtgggaggacctggccacaaggccagggtgctggccgaggccatgagccaggtgaccaactctgccaccatcatgatgcagagaggcaacttccggaaccagagaaagaccgtgaagtgcttcaactgtggcaaagagggacacattgccaagaactgcagggctcccaggaagaaaggctgctggaagtgcggaaaagaaggccaccagatgaaggactgcaccgagaggcaggccaacttcctgggcaagatctggcctagcaacaagggcaggcctggcaacttcctgcagaacagacccgagcccaccgctcctcccgaggaaagcttccggtttggcgaggaaaccaccacccctagccagaagcaggaacccatcgacaaagagatgtaccctctggccagcctgaagagcctgttcggcaacgaccccagcagccagatggctcccatcagcccaatcgagacagtgcctgtgaagctgaagcctggcatggacggacccagggtgaagcagtggcctctgaccgaggaaaagatcaaagccctgacagccatctgcgaggaaatggaaaaagagggcaagatcaccaagatcggacccgagaacccctacaacacccctgtgttcgccatcaagaagaaagacagcaccaagtggaggaaactggtggacttcagagagctgaacaagcggacccaggacttctgggaggtgcagctgggcatccctcaccctgctggcctgaagaaaaagaaaagcgtgaccgtgctggctgtgggagatgcctacttcagcgtgcctctggacgagggcttccggaagtacacagccttcaccatccccagcaccaacaacgagacacctggcatcagataccagtacaacgtgctgcctcagggctggaaaggcagccctgccatcttccagtgcagcatgaccagaatcctggaacccttcagagccaagaaccctgagatcgtgatctaccagtatatggctgccctctacgtgggcagcgacctggaaatcggacagcacagagccaaaatcgaagaactccgcgagcacctgctgaagtggggattcaccacccctgacaagaagcaccagaaagagcctcccttcctgtggatgggctacgagctgcaccctgacaagtggaccgtgcagcccatccagctgccagagaaggactcctggaccgtgaacgacatccagaaactggtcggcaagctgaactgggccagccagatctaccctggcatcaaagtcagacagctgtgtaagctgctgaggggagccaaagcactgaccgacatcgtgcctctgacagaagaagccgagctggaactggccgagaacagagagatcctgaaagaacccgtgcacggagtgtactacgacccctccaaggacctgattgccgagatccagaaacagggacacgaccagtggacctaccagatctatcaggaacctttcaagaacctgaaaacaggcaagtacgccaagatgcggacagcccacaccaacgacgtgaagcagctgaccgaagccgtgcagaaaatcgccatggaaagcatcgtgatctggggaaagacacccaagttcaggctgcccatccagaaagagacatgggaaacctggtggaccgactactggcaggccacctggattcccgagtgggagttcgtgaacaccccacccctggtgaagctgtggtatcagctggaaaaggaccctatcgctggcgtggagacattctacgtggctggagctgccaacagagagacaaagctgggcaaggctggctacgtgaccgacagaggcagacagaaaatcgtgagcctgaccgaaaccaccaaccagaaaacagccctgcaggccatctatctggcactgcaggacagcggaagcgaggtgaacatcgtgacagccagccagtatgccctgggcatcatccaggcccagcctgacaagagcgagagcgagctggtgaaccagatcatcgagcagctgatcaagaaagaacgggtgtacctgagctgggtgccagcccacaagggcatcggagggaacgagcaggtggacaagctggtgtccagcggaatccggaaggtgctgttcctggacggcatcgataaagcccaggaagagcacgagaagtaccacagcaattggagagccatggccagcgacttcaacctgcctcccgtggtggccaaagaaatcgtggccagctgcgaccagtgccagctgaaaggcgaggccatgcacggacaggtggactgctcccctggcatctggcagctggcatgcacccacctggaaggcaagatcattctggtggccgtgcacgtggccagcggatacatcgaagccgaagtgatccctgccgagacagggcaggaaacagcctacttcatcctgaagctggctggcagatggcctgtgaaggtgatccacacagccaacggcagcaacttcacctctgctgccgtgaaggctgcctgttggtgggctggcattcagcaggaatttggcatcccctacaatccccagtctcagggagtggtggccagcatgaacaaagagctgaagaagatcatcggacaggtcagggatcaggccgagcacctgaaaactgccgtccagatggccgtgttcatccacaacttcaagcggaagggagggatcggagggtactctgctggcgagcggatcatcgacatcattgccaccgatatccagaccaaagagctgcagaaacagatcatcaagatccagaacttcagggtgtactacagggacagcagggaccccatctggaagggacctgccaagctgctgtggaaaggcgaaggagccgtcgtcatccaggacaacagcgacatcaaggtggtgcccagacggaaggtgaaaatcatcaaggactacggcaaacagatggctggagccgactgtgtcgctggcaggcaggacgaggac

SEQ ID NO: 21 - DNA, 4023 bp, Artificial Sequence
  nucleotide sequence encoding mos2GagPol
atgggagccagagccagcatcctgcgaggagggaagctggacaagtgggagaagatcaggctgaggcctggagggaagaaacactacatgctgaagcacctggtctgggccagcagagagctggaacggtttgccctcaatcctggcctgctggaaaccagcgagggctgcaagcagatcatcaagcagctgcagcctgccctgcagacaggcaccgaggaactgcggagcctgttcaacaccgtggccaccctgtactgcgtgcatgccgagatcgaagtgagggacaccaaagaagccctggacaagatcgaggaagagcagaacaagagccagcagaaaacccagcaggccaaagaagccgacggcaaggtctcccagaactaccccatcgtgcagaacctgcagggacagatggtgcaccagcccatcagccctcggacactgaatgcctgggtgaaggtgatcgaggaaaaggccttcagccctgaggtgatccccatgttcacagccctgagcgagggagccacaccccaggacctgaacaccatgctgaacaccgtgggagggcaccaggctgccatgcagatgctgaaggacaccatcaacgaggaagctgccgagtgggacaggctgcaccctgtgcacgctggacctgtggctcctggccagatgagagagcccagaggcagcgatattgctggcaccacctccaatctgcaggaacagatcgcctggatgaccagcaaccctcccatccctgtgggagacatctacaagcggtggatcatcctgggactgaacaagatcgtgcggatgtacagccctacctccatcctggacatcaagcagggacccaaagagcctttcagggactacgtggaccggttcttcaagaccctgagagccgagcaggccacccaggacgtgaagaactggatgaccgacaccctgctggtgcagaacgccaaccctgactgcaagaccatcctgagagccctgggacctggagccaccctggaagagatgatgacagcctgccagggagtgggaggaccctctcacaaggctagggtgctggccgaggccatgagccagaccaacagcaccatcctgatgcagcggagcaacttcaagggcagcaagcggatcgtgaagtgcttcaactgtggcaaagagggacacattgccagaaactgtagggcacccaggaagaaaggctgctggaagtgcggaaaagaaggccaccagatgaaggactgcaccgagaggcaggccaacttcctgggcaagatctggcctagccacaagggcagacctggcaacttcctgcagagcagacccgagcccaccgctcctccagccgagagcttccggttcgaggaaaccacccctgctcccaagcaggaacctaaggacagagagcctctgaccagcctgagaagcctgttcggcagcgaccctctgagccagatggctcccatctcccctatcgagacagtgcctgtgaagctgaagcctggcatggacggacccaaggtgaaacagtggcctctgaccgaggaaaagatcaaagccctggtggagatctgtaccgagatggaaaaagagggcaagatcagcaagatcggacccgagaacccctacaacacccctatcttcgccatcaagaagaaagacagcaccaagtggaggaaactggtggacttcagagagctgaacaagcggacccaggacttctgggaggtgcagctgggcatccctcaccctgctggcctgaagaaaaagaaaagcgtgaccgtgctggccgtgggagatgcctacttcagcgtgcctctggacgaggacttcagaaagtacacagccttcaccatccccagcatcaacaacgagacacctggcatcagataccagtacaacgtgctgcctcagggatggaagggctctcctgcaatcttccagagcagcatgaccaagatcctggaacccttccggaagcagaaccctgacatcgtgatctaccagtacatggcagccctgtacgtcggcagcgacctggaaatcggacagcaccggaccaagatcgaagaactcaggcagcacctgctgcggtggggattcaccacccctgacaagaagcaccagaaagagcctcccttcctgtggatgggctacgagctgcacccagacaagtggaccgtgcagcccatcgtgctgcctgagaaggactcctggaccgtgaacgacatccagaaactggtcggcaagctgaactgggccagccagatctacgctggcatcaaagtgaagcagctgtgtaagctcctgagaggcaccaaagccctgaccgaggtggtgccactgacagaggaagccgagctggaactggccgagaacagagagatcctgaaagaacccgtgcacggagtgtactacgaccccagcaaggacctgattgccgagatccagaagcagggacagggacagtggacctaccagatctaccaggaacccttcaagaacctgaaaacaggcaagtacgccaggatgaggggagcccacaccaacgacgtcaaacagctgaccgaagccgtgcagaagatcgccaccgagagcatcgtgatttggggaaagacacccaagttcaagctgcccatccagaaagagacatgggaggcctggtggaccgagtactggcaggccacctggattcccgagtgggagttcgtgaacaccccacccctggtgaagctgtggtatcagctggaaaaagaacccatcgtgggagccgagacattctacgtggctggagctgccaacagagagacaaagctgggcaaggctggctacgtgaccgacagaggcaggcagaaagtggtgtccctgaccgataccaccaaccagaaaacagccctgcaggccatccacctggctctgcaggactctggcctggaagtgaacatcgtgacagccagccagtatgccctgggcatcattcaggcacagcctgacaagagcgagagcgagctggtgtctcagatcattgagcagctgatcaagaaagaaaaggtgtacctggcctgggtgccagcccacaaggggatcggagggaacgagcaggtggacaagctggtgtccaggggcatccggaaggtgctgtttctggacggcatcgacaaagcccaggaagagcacgagaagtaccacagcaattggagagccatggccagcgagttcaacctgcctcccatcgtggccaaagaaatcgtggcctcttgcgacaagtgccagctgaaaggcgaggccattcacggacaggtggactgcagcccaggcatctggcagctggcctgcacccacctggaaggcaaggtgatcctggtggccgtgcacgtggcctctggatacatcgaagccgaagtgatccctgccgagacaggccaggaaacagcctacttcctgctgaagctggctggcaggtggcctgtgaaaaccatccacacagccaacggcagcaacttcacctctgccaccgtgaaggctgcctgttggtgggctggcattaagcaggaatttggcatcccctacaaccctcagtctcagggagtggtggcctccatcaacaaagagctgaagaagatcatcggacaggtcagggatcaggccgagcatctgaaaacagccgtccagatggccgtgttcatccacaacttcaagcggaagggagggatcggagagtactctgctggcgagaggatcgtggacattatcgccagcgatatccagaccaaagaactgcagaagcagatcacaaagatccagaacttcagggtgtactacagggacagcagagatcccctgtggaagggacctgccaagctgctgtggaaaggcgaaggagccgtcgtcatccaggacaacagcgacatcaaggtggtgcccagacggaaggccaagatcatcagagactacggcaaacagatggctggcgacgactgcgtcgcctctaggcaggacgaggac

SEQ ID NO: 22 - DNA, 2055 bp, Artificial Sequence
  nucleotide sequence encoding mos1Env
atgcgggtgaccggcatccggaagaactaccagcacctgtggcggtggggcaccatgctgctgggcatcctgatgatttgctctgccgccggaaagctgtgggtgaccgtgtactacggcgtgcccgtgtggaaagaggccaccaccaccctgttctgcgccagcgacgccaaggcctacgacaccgaggtgcacaacgtgtgggccacccacgcctgcgtgcccaccgaccccaacccccaggaagtggtcctggaaaacgtgaccgagaacttcaacatgtggaagaacaacatggtggagcagatgcacgaggacatcatcagcctgtgggaccagagcctgaagccctgcgtgaagctgacccccctgtgcgtgaccctgaactgcaccgacgacgtgcggaacgtgaccaacaacgccaccaacaccaacagcagctggggcgagcctatggaaaagggcgagatcaagaactgcagcttcaacatcaccacctccatccggaacaaggtgcagaagcagtacgccctgttctacaagctggacgtggtgcccatcgacaacgacagcaacaacaccaactaccggctgatcagctgcaacaccagcgtgatcacccaggcctgccccaaggtgtccttcgagcccatccccatccactactgcgcccctgccggcttcgccatcctgaagtgcaacgacaagaagttcaacggcaccggcccctgcaccaacgtgagcaccgtgcagtgcacccacggcatccggcccgtggtgtccacccagctgctgctgaacggcagcctggccgaggaagaggtggtgatcagaagcgagaatttcaccaacaatgccaagaccatcatggtgcagctgaacgtgagcgtggagatcaactgcacccggcccaacaacaacacccggaagagcatccacatcggccctggcagggccttctacacagccggcgacatcatcggcgacatccggcaggcccactgcaacatcagccgggccaactggaacaacaccctgcggcagatcgtggagaagctgggcaagcagttcggcaacaacaagaccatcgtgttcaaccacagcagcggcggagaccccgagatcgtgatgcacagcttcaactgtggcggcgagttcttctactgcaacagcaccaagctgttcaacagcacctggacctggaacaactccacctggaataacaccaagcggagcaacgacaccgaagagcacatcaccctgccctgccggatcaagcagattatcaatatgtggcaggaggtcggcaaggccatgtacgcccctcccatccggggccagatccggtgcagcagcaacatcaccggcctgctgctgacccgggacggcggcaacgataccagcggcaccgagatcttccggcctggcggcggagatatgcgggacaactggcggagcgagctgtacaagtacaaggtggtgaagatcgagcccctgggcgtggctcccaccaaggccaagcggcgggtggtgcagagcgagaagagcgccgtgggcatcggcgccgtgtttctgggcttcctgggagccgccggaagcaccatgggagccgccagcatgaccctgaccgtgcaggcccggctgctgctgtccggcatcgtgcagcagcagaacaacctgctccgggccatcgaggcccagcagcacctgctgcagctgaccgtgtggggcatcaagcagctgcaggccagggtgctggccgtggagagatacctgaaggatcagcagctcctggggatctggggctgcagcggcaagctgatctgcaccaccaccgtgccctggaacgccagctggtccaacaagagcctggacaagatctggaacaatatgacctggatggaatgggagcgcgagatcaacaattacaccagcctgatctacaccctgatcgaggaaagccagaaccagcaggaaaagaacgagcaggaactgctggaactggacaagtgggccagcctgtggaactggttcgacatcagcaactggctgtgg

SEQ ID NO: 23 - DNA, 2052 bp, Artificial Sequence
  nucleotide sequence encoding mos2Env
atgagagtgcggggcatccagcggaactggccccagtggtggatctggggcatcctgggcttttggatgatcatcatctgccgggtgatgggcaacctgtgggtgaccgtgtactacggcgtgcccgtgtggaaagaggccaagaccaccctgttctgcgccagcgacgccaaggcctacgagaaagaggtgcacaacgtgtgggccacccacgcctgcgtgcccaccgaccccaacccccaggaaatggtcctggaaaacgtgaccgagaacttcaacatgtggaagaacgacatggtggaccagatgcacgaggacatcatccggctgtgggaccagagcctgaagccctgcgtgaagctgacccccctgtgcgtgaccctggaatgccggaacgtgagaaacgtgagcagcaacggcacctacaacatcatccacaacgagacctacaaagagatgaagaactgcagcttcaacgccaccaccgtggtggaggaccggaagcagaaggtgcacgccctgttctaccggctggacatcgtgcccctggacgagaacaacagcagcgagaagtccagcgagaacagctccgagtactaccggctgatcaactgcaacaccagcgccatcacccaggcctgccccaaggtgtccttcgaccccatccccatccactactgcgcccctgccggctacgccatcctgaagtgcaacaacaagaccttcaacggcaccggcccctgcaacaacgtgagcaccgtgcagtgcacccacggcatcaagcccgtggtgtccacccagctgctgctgaacggcagcctggccgaggaagagatcatcatccggtccgagaacctgaccaacaacgccaagaccatcatcgtgcacctgaatgagaccgtgaacatcacctgcacccggcccaacaacaacacccggaagagcatccggatcggccctggccagaccttttacgccaccggcgacatcatcggcgacatccggcaggcccactgcaacctgagccgggacggctggaacaagaccctgcagggcgtgaagaagaagctggccgagcacttccccaataagaccatcaacttcaccagcagcagcggcggagacctggaaatcaccacccacagcttcaactgcaggggcgagttcttctactgcaatacctccggcctgttcaatggcacctacatgcccaacggcaccaacagcaacagcagcagcaacatcaccctgccctgccggatcaagcagatcatcaatatgtggcaggaggtcggcagggccatgtacgcccctcccatcgccggcaatatcacctgccggtccaacatcaccggcctgctgctgaccagggacggcggcagcaacaacggcgtgcctaacgacaccgagaccttccggcctggcggcggagatatgcggaacaactggcggagcgagctgtacaagtacaaggtggtggaggtgaagcccctgggcgtggctcctaccgaggccaagcggcgggtggtggagagcgagaagagcgccgtgggcatcggcgccgtgtttctgggcattctgggagccgccggaagcaccatgggagccgccagcatcaccctgaccgtgcaggcccggcagctgctgtccggcatcgtgcagcagcagagcaacctgctgagagccatcgaggcccagcagcacatgctgcagctgaccgtgtggggcatcaagcagctgcagacccgggtgctggccatcgagagatacctgcaggatcagcagctcctgggcctgtggggctgcagcggcaagctgatctgcaccaccgccgtgccctggaacaccagctggtccaacaagagccagaccgacatctgggacaacatgacctggatgcagtgggacaaagagatcggcaactacaccggcgagatctacaggctgctggaagagagccagaaccagcaggaaaagaacgagaaggacctgctggccctggacagctggaagaacctgtggaactggttcgacatcaccaactggctgtgg

SEQ ID NO: 24 - DNA, 829 bp, Artificial Sequence
  CMV promoter used for expression of antigens in Ad26 vectors
tcaatattggccattagccatattattcattggttatatagcataaatcaatattggctattggccattgcatacgttgtatccatatcataatatgtacatttatattggctcatgtccaacattaccgccatgttgacattgattattgactagttattaatagtaatcaattacggggtcattagttcatagcccatatatggagttccgcgttacataacttacggtaaatggcccgcctggctgaccgcccaacgacccccgcccattgacgtcaataatgacgtatgttcccatagtaacgccaatagggactttccattgacgtcaatgggtggagtatttacggtaaactgcccacttggcagtacatcaagtgtatcatatgccaagtacgccccctattgacgtcaatgacggtaaatggcccgcctggcattatgcccagtacatgaccttatgggactttcctacttggcagtacatctacgtattagtcatcgctattaccatggtgatgcggttttggcagtacatcaatgggcgtggatagcggtttgactcacggggatttccaagtctccaccccattgacgtcaatgggagtttgttttggcaccaaaatcaacgggactttccaaaatgtcgtaacaactccgccccattgacgcaaatgggcggtaggcgtgtacggtgggaggtctatataagcagagctcgtttagtgaaccgtcagatcgcctggagacgccatccacgctgttttgacctccatagaagacaccgggaccgatccagcctccgcggccgggaacggtgcattgga

SEQ ID NO: 25 - DNA, 2586 bp, Artificial Sequence
  nucleotide sequence encoding c4
atgagagtgcggggcatgctgagaaactggcagcagtggtggatctggtccagcctgggcttctggatgctgatgatctacagcgtgatgggcaacctgtgggtcaccgtgtactacggcgtgcccgtgtggaaggacgccaagaccaccctgttttgcgcctccgatgccaaggcctacgagaaagaggtgcacaacgtctgggccacccacgcctgtgtgcccaccgaccccaatccccaggaaatcgtcctgggcaacgtgaccgagaacttcaacatgtggaagaacgacatggtcgatcagatgcacgaggacatcatctccctgtgggacgcctccctggaaccctgcgtgaagctgacccctctgtgcgtgaccctgaactgccggaacgtgcgcaacgtgtccagcaacggcacctacaacatcatccacaacgagacatacaaagagatgaagaactgcagcttcaacgctaccaccgtggtcgaggaccggaagcagaaggtgcacgccctgttctaccggctggacatcgtgcccctggacgagaacaacagcagcgagaagtcctccgagaacagctccgagtactacagactgatcaactgcaacaccagcgccatcacccaggcctgccccaaggtgtccttcgaccctatccccatccactactgcgcccctgccggctacgccatcctgaagtgcaacaacaagaccttcaatggcaccggcccctgcaacaatgtgtccaccgtgcagtgcacccacggcatcaagcccgtggtgtctacccagctgctgctgaacggcagcctggccgaggaagagatcattatcagaagcgagaacctgaccaacaacgccaaaaccatcatcgtccacctgaacgaaaccgtgaacatcacctgtacccggcctaacaacaacacccggaagtccatccggatcggccctggccagaccttttacgccaccggcgatattatcggcgacatccggcaggcccactgcaatctgagccgggacggctggaacaagacactgcagggcgtcaagaagaagctggccgaacacttccctaacaagactatcaagttcgcccctcactctggcggcgacctggaaatcaccacccacaccttcaactgtcggggcgagttcttctactgcaatacctccaacctgttcaacgagagcaacatcgagcggaacgacagcatcatcacactgccttgccggatcaagcagattatcaatatgtggcaggaagtgggcagagccatctacgcccctccaatcgccggcaacatcacatgccggtccaatatcaccggcctgctgctcaccagagatggcggctccaacaatggcgtgccaaacgacaccgagacattcagacccggcggaggcgacatgcggaacaattggcggagcgagctgtacaagtacaaggtggtggaagtgaagcccctgggcgtggcccctaccgaggccaagagaagagtggtcgaacgcgagaagcgggccgtgggaatcggagccgtgtttctgggaatcctgggagccgctggctctaccatgggcgctgcctctatcaccctgacagtgcaggccagacagctgctcagcggcatcgtgcagcagcagagcaacctgctgagagccattgaggcccagcagcacatgctgcagctgaccgtgtggggcattaagcagctccagacacgggtgctggccatcgagagatacctgcaggatcagcagctcctgggcctgtggggctgtagcggcaagctgatctgtaccaccgccgtgccctggaatacctcttggagcaacaagagccagaccgacatctgggacaacatgacctggatgcagtgggacaaagaaatcggcaactataccggcgagatctatagactgctggaagagtcccagaaccagcaggaaaagaacgagaaggacctgctggccctggattcttggaacaatctgtggaactggttcagcatctccaagtggctgtggtacatcaagatcttcatcatgatcgtgggcggcctgatcggcctgcggatcatctttgccgtgctgagcatcgtgaaccgcgtgcggcagggatacagccctctgagcctgcagaccctgactcagaaccctggcggactggacagactgggccggattgaggaagaaggcggcgagcaggacaaggatcggagcatcaggctggtcaacggcttcttcgctctgttttgggacgacctgcggagcctgtgcctgttcagctaccacagactgcgggactttatcctgattgtggccagagccgtcgaactgctggggagaagctctctgagaggcctgcagcggggctgggagattctgaagtacctgggctccctgctgcagtactggggcctggaactgaagaagtctgccatcaatctgctcgacacaatcgctattgccgtggccgaaggcaccgatagaatcatcgagctgatccagcggatctgccgggccatctgcaacatccccagacggatcagacagggcttcgaggccgctctgcag

SEQ ID NO: 26 - DNA, 2133 bp, Artificial Sequence
  nucleotide sequence encoding C4D7
atgagagtgcggggcatgctgagaaactggcagcagtggtggatctggtccagcctgggcttctggatgctgatgatctacagcgtgatgggcaacctgtgggtcaccgtgtactacggcgtgcccgtgtggaaggacgccaagaccaccctgttttgcgcctccgatgccaaggcctacgagaaagaggtgcacaacgtctgggccacccacgcctgtgtgcccaccgaccccaatccccaggaaatcgtcctgggcaacgtgaccgagaacttcaacatgtggaagaacgacatggtcgatcagatgcacgaggacatcatctccctgtgggacgcctccctggaaccctgcgtgaagctgacccctctgtgcgtgaccctgaactgccggaacgtgcgcaacgtgtccagcaacggcacctacaacatcatccacaacgagacatacaaagagatgaagaactgcagcttcaacgctaccaccgtggtcgaggaccggaagcagaaggtgcacgccctgttctaccggctggacatcgtgcccctggacgagaacaacagcagcgagaagtcctccgagaacagctccgagtactacagactgatcaactgcaacaccagcgccatcacccaggcctgccccaaggtgtccttcgaccctatccccatccactactgcgcccctgccggctacgccatcctgaagtgcaacaacaagaccttcaatggcaccggcccctgcaacaatgtgtccaccgtgcagtgcacccacggcatcaagcccgtggtgtctacccagctgctgctgaacggcagcctggccgaggaagagatcattatcagaagcgagaacctgaccaacaacgccaaaaccatcatcgtccacctgaacgaaaccgtgaacatcacctgtacccggcctaacaacaacacccggaagtccatccggatcggccctggccagaccttttacgccaccggcgatattatcggcgacatccggcaggcccactgcaatctgagccgggacggctggaacaagacactgcagggcgtcaagaagaagctggccgaacacttccctaacaagactatcaagttcgcccctcactctggcggcgacctggaaatcaccacccacaccttcaactgtcggggcgagttcttctactgcaatacctccaacctgttcaacgagagcaacatcgagcggaacgacagcatcatcacactgccttgccggatcaagcagattatcaatatgtggcaggaagtgggcagagccatctacgcccctccaatcgccggcaacatcacatgccggtccaatatcaccggcctgctgctcaccagagatggcggctccaacaatggcgtgccaaacgacaccgagacattcagacccggcggaggcgacatgcggaacaattggcggagcgagctgtacaagtacaaggtggtggaagtgaagcccctgggcgtggcccctaccgaggccaagagaagagtggtcgaacgcgagaagcgggccgtgggaatcggagccgtgtttctgggaatcctgggagccgctggctctaccatgggcgctgcctctatcaccctgacagtgcaggccagacagctgctcagcggcatcgtgcagcagcagagcaacctgctgagagccattgaggcccagcagcacatgctgcagctgaccgtgtggggcattaagcagctccagacacgggtgctggccatcgagagatacctgcaggatcagcagctcctgggcctgtggggctgtagcggcaagctgatctgtaccaccgccgtgccctggaatacctcttggagcaacaagagccagaccgacatctgggacaacatgacctggatgcagtgggacaaagaaatcggcaactataccggcgagatctatagactgctggaagagtcccagaaccagcaggaaaagaacgagaaggacctgctggccctggattcttggaacaatctgtggaactggttcagcatctccaagtggctgtggtacatcaagatcttcatcatgatcgtgggcggcctgatcggcctgcggatcatctttgccgtgctgagcatcgtgaaccgcgtgcggcagggctac

SEQ ID NO: 27 - DNA, 2112 bp, Artificial Sequence
  nucleotide sequence encoding sC4
atgagagtgcggggcatgctgagaaactggcagcagtggtggatctggtccagcctgggcttctggatgctgatgatctacagcgtgatgggcaacctgtgggtcaccgtgtactacggcgtgcccgtgtggaaggacgccaagaccaccctgttttgcgcctccgatgccaaggcctacgagaaagaggtgcacaacgtctgggccacccacgcctgtgtgcccaccgaccccaatccccaggaaatcgtcctgggcaacgtgaccgagaacttcaacatgtggaagaacgacatggtcgatcagatgcacgaggacatcatctccctgtgggacgcctccctggaaccctgcgtgaagctgacccctctgtgcgtgaccctgaactgccggaacgtgcgcaacgtgtccagcaacggcacctacaacatcatccacaacgagacatacaaagagatgaagaactgcagcttcaacgctaccaccgtggtcgaggaccggaagcagaaggtgcacgccctgttctaccggctggacatcgtgcccctggacgagaacaacagcagcgagaagtcctccgagaacagctccgagtactacagactgatcaactgcaacaccagcgccatcacccaggcctgccccaaggtgtccttcgaccctatccccatccactactgcgcccctgccggctacgccatcctgaagtgcaacaacaagaccttcaatggcaccggcccctgcaacaatgtgtccaccgtgcagtgcacccacggcatcaagcccgtggtgtctacccagctgctgctgaacggcagcctggccgaggaagagatcattatcagaagcgagaacctgaccaacaacgccaaaaccatcatcgtccacctgaacgaaaccgtgaacatcacctgtacccggcctaacaacaacacccggaagtccatccggatcggccctggccagaccttttacgccaccggcgatattatcggcgacatccggcaggcccactgcaatctgagccgggacggctggaacaagacactgcagggcgtcaagaagaagctggccgaacacttccctaacaagactatcaagttcgcccctcactctggcggcgacctggaaatcaccacccacaccttcaactgtcggggcgagttcttctactgcaatacctccaacctgttcaacgagagcaacatcgagcggaacgacagcatcatcacactgccttgccggatcaagcagattatcaatatgtggcaggaagtgggcagagccatctacgcccctccaatcgccggcaacatcacatgccggtccaatatcaccggcctgctgctcaccagagatggcggctccaacaatggcgtgccaaacgacaccgagacattcagacccggcggaggcgacatgcggaacaattggcggagcgagctgtacaagtacaaggtggtggaagtgaagcccctgggcgtggcccctaccgaggccaagagaagagtggtcgaacgcgaggaacgggccgtgggaatcggagccgtgtttctgggaatcctgggagccgctggctctaccatgggcgctgcctctatcaccctgacagtgcaggccagacagctgctcagcggcatcgtgcagcagcagagcaacctgctgagagccattgaggcccagcagcacatgctgcagctgaccgtgtggggcattaagcagctccagacacgggtgctggccatcgagagatacctgcaggatcagcagctcctgggcctgtggggctgtagcggcaagctgatctgtaccaccgccgtgccctggaatacctcttggagcaacaagagccagaccgacatctgggacaacatgacctggatgcagtgggacaaagaaatcggcaactataccggcgagatctatagactgctggaagagtcccagaaccagcaggaaaagatgaagcagatcgaggacaagatcgaagagattctgagcaagatctaccacatcgagaacgagatcgcccgcatcaagaaactgatcggcgaagtgggatccggcgctcccacaaaggccaaaagacgggtggtgcagcgcgagaaacgc

SEQ ID NO: 28 - protein, 1350 aa, Artificial Sequence
  mos1GagPol mosaic antigen sequence
MGARASVLSGGELDRWEKIRLRPGGKKKYRLKHIVWASRELERFAVNPGLLETSEGCRQILGQLQPSLQTGSEELRSLYNTVATLYCVHQRIEIKDTKEALEKIEEEQNKSKKKAQQAAADTGNSSQVSQNYPIVQNIQGQMVHQAISPRTLNAWVKVVEEKAFSPEVIPMFSALSEGATPQDLNTMLNTVGGHQAAMQMLKETINEEAAEWDRVHPVHAGPIAPGQMREPRGSDIAGTTSTLQEQIGWMTNNPPIPVGEIYKRWIILGLNKIVRMYSPVSILDIRQGPKEPFRDYVDRFYKTLRAEQASQDVKNWMTETLLVQNANPDCKTILKALGPAATLEEMMTACQGVGGPGHKARVLAEAMSQVTNSATIMMQRGNFRNQRKTVKCFNCGKEGHIAKNCRAPRKKGCWKCGKEGHQMKDCTERQANFLGKIWPSNKGRPGNFLQNRPEPTAPPEESFRFGEETTTPSQKQEPIDKEMYPLASLKSLFGNDPSSQMAPISPIETVPVKLKPGMDGPRVKQWPLTEEKIKALTAICEEMEKEGKITKIGPENPYNTPVFAIKKKDSTKWRKLVDFRELNKRTQDFWEVQLGIPHPAGLKKKKSVTVLAVGDAYFSVPLDEGFRKYTAFTIPSTNNETPGIRYQYNVLPQGWKGSPAIFQCSMTRILEPFRAKNPEIVIYQYMAALYVGSDLEIGQHRAKIEELREHLLKWGFTTPDKKHQKEPPFLWMGYELHPDKWTVQPIQLPEKDSWTVNDIQKLVGKLNWASQIYPGIKVRQLCKLLRGAKALTDIVPLTEEAELELAENREILKEPVHGVYYDPSKDLIAEIQKQGHDQWTYQIYQEPFKNLKTGKYAKMRTAHTNDVKQLTEAVQKIAMESIVIWGKTPKFRLPIQKETWETWWTDYWQATWIPEWEFVNTPPLVKLWYQLEKDPIAGVETFYVAGAANRETKLGKAGYVTDRGRQKIVSLTETTNQKTALQAIYLALQDSGSEVNIVTASQYALGIIQAQPDKSESELVNQIIEQLIKKERVYLSWVPAHKGIGGNEQVDKLVSSGIRKVLFLDGIDKAQEEHEKYHSNWRAMASDFNLPPVVAKEIVASCDQCQLKGEAMHGQVDCSPGIWQLACTHLEGKIILVAVHVASGYIEAEVIPAETGQETAYFILKLAGRWPVKVIHTANGSNFTSAAVKAACWWAGIQQEFGIPYNPQSQGVVASMNKELKKIIGQVRDQAEHLKTAVQMAVFIHNFKRKGGIGGYSAGERIIDIIATDIQTKELQKQIIKIQNFRVYYRDSRDPIWKGPAKLLWKGEGAVVIQDNSDIKVVPRRKVKIIKDYGKQMAGADCVAGRQDED

SEQ ID NO: 29 - protein, 1341 aa, Artificial Sequence
  mos2GagPol mosaic antigen sequence
MGARASILRGGKLDKWEKIRLRPGGKKHYMLKHLVWASRELERFALNPGLLETSEGCKQIIKQLQPALQTGTEELRSLFNTVATLYCVHAEIEVRDTKEALDKIEEEQNKSQQKTQQAKEADGKVSQNYPIVQNLQGQMVHQPISPRTLNAWVKVIEEKAFSPEVIPMFTALSEGATPQDLNTMLNTVGGHQAAMQMLKDTINEEAAEWDRLHPVHAGPVAPGQMREPRGSDIAGTTSNLQEQIAWMTSNPPIPVGDIYKRWIILGLNKIVRMYSPTSILDIKQGPKEPFRDYVDRFFKTLRAEQATQDVKNWMTDTLLVQNANPDCKTILRALGPGATLEEMMTACQGVGGPSHKARVLAEAMSQTNSTILMQRSNFKGSKRIVKCFNCGKEGHIARNCRAPRKKGCWKCGKEGHQMKDCTERQANFLGKIWPSHKGRPGNFLQSRPEPTAPPAESFRFEETTPAPKQEPKDREPLTSLRSLFGSDPLSQMAPISPIETVPVKLKPGMDGPKVKQWPLTEEKIKALVEICTEMEKEGKISKIGPENPYNTPIFAIKKKDSTKWRKLVDFRELNKRTQDFWEVQLGIPHPAGLKKKKSVTVLAVGDAYFSVPLDEDFRKYTAFTIPSINNETPGIRYQYNVLPQGWKGSPAIFQSSMTKILEPFRKQNPDIVIYQYMAALYVGSDLEIGQHRTKIEELRQHLLRWGFTTPDKKHQKEPPFLWMGYELHPDKWTVQPIVLPEKDSWTVNDIQKLVGKLNWASQIYAGIKVKQLCKLLRGTKALTEVVPLTEEAELELAENREILKEPVHGVYYDPSKDLIAEIQKQGQGQWTYQIYQEPFKNLKTGKYARMRGAHTNDVKQLTEAVQKIATESIVIWGKTPKFKLPIQKETWEAWWTEYWQATWIPEWEFVNTPPLVKLWYQLEKEPIVGAETFYVAGAANRETKLGKAGYVTDRGRQKVVSLTDTTNQKTALQAIHLALQDSGLEVNIVTASQYALGIIQAQPDKSESELVSQIIEQLIKKEKVYLAWVPAHKGIGGNEQVDKLVSRGIRKVLFLDGIDKAQEEHEKYHSNWRAMASEFNLPPIVAKEIVASCDKCQLKGEAIHGQVDCSPGIWQLACTHLEGKVILVAVHVASGYIEAEVIPAETGQETAYFLLKLAGRWPVKTIHTANGSNFTSATVKAACWWAGIKQEFGIPYNPQSQGVVASINKELKKIIGQVRDQAEHLKTAVQMAVFIHNFKRKGGIGEYSAGERIVDIIASDIQTKELQKQITKIQNFRVYYRDSRDPLWKGPAKLLWKGEGAVVIQDNSDIKVVPRRKAKIIRDYGKQMAGDDCVASRQDED

SEQ ID NO: 30 - protein, 709 aa, Artificial Sequence
  sc1 sequence
MRVRGIQRNWPQWWIWGILGFWMIIICRVMGNLWVTVYYGVPVWKEAKTTLFCASDAKAYEKEVHNVWATHACVPTDPNPQEMVLENVTENFNMWKNDMVDQMHEDIIRLWDQSLKPCVKLTPLCVTLECRNVRNVSSNGTYNIIHNETYKEMKNCSFNATTVVEDRKQKVHALFYRLDIVPLDENNSSEKSSENSSEYYRLINCNTSAITQACPKVSFDPIPIHYCAPAGYAILKCNNKTFNGTGPCNNVSTVQCTHGIKPVVSTQLLLNGSLAEEEIIIRSENLTNNAKTIIVHLNETVNITCTRPNNNTRKSIRIGPGQTFYATGDIIGDIRQAHCNLSRDGWNKTLQGVKKKLAEHFPNKTINFTSSSGGDLEITTHSFNCRGEFFYCNTSGLFNGTYMPNGTNSNSSSNITLPCRIKQIINMWQEVGRAMYAPPIAGNITCRSNITGLLLTRDGGSNNGVPNDTETFRPGGGDMRNNWRSELYKYKVVEVKPLGVAPTEAKRRVVEREERAVGIGAVFLGILGAAGSTMGAASITLTVQARQLLSGIVQQQSNLLRAIEAQQHMLQLTVWGIKQLQTRVLAIERYLQDQQLLGLWGCSGKLICTTAVPWNTSWSNKSQTDIWDNMTWMQWDKEIGNYTGEIYRLLEESQNQQEKMKQIEDKIEEILSKIYHIENEIARIKKLIGEVGSGAPTKAKRRVVQREKR

SEQ ID NO: 31 - protein, 867 aa, Artificial Sequence
  C1 sequence
MRVRGIQRNWPQWWIWGILGFWMIIICRVMGNLWVTVYYGVPVWKEAKTTLFCASDAKAYEKEVHNVWATHACVPTDPNPQEMVLENVTENFNMWKNDMVDQMHEDIIRLWDQSLKPCVKLTPLCVTLECRNVRNVSSNGTYNIIHNETYKEMKNCSFNATTVVEDRKQKVHALFYRLDIVPLDENNSSEKSSENSSEYYRLINCNTSAITQACPKVSFDPIPIHYCAPAGYAILKCNNKTFNGTGPCNNVSTVQCTHGIKPVVSTQLLLNGSLAEEEIIIRSENLTNNAKTIIVHLNETVNITCTRPNNNTRKSIRIGPGQTFYATGDIIGDIRQAHCNLSRDGWNKTLQGVKKKLAEHFPNKTINFTSSSGGDLEITTHSFNCRGEFFYCNTSGLFNGTYMPNGTNSNSSSNITLPCRIKQIINMWQEVGRAMYAPPIAGNITCRSNITGLLLTRDGGSNNGVPNDTETFRPGGGDMRNNWRSELYKYKVVEVKPLGVAPTEAKRRVVEREKRAVGIGAVFLGILGAAGSTMGAASITLTVQARQLLSGIVQQQSNLLRAIEAQQHMLQLTVWGIKQLQTRVLAIERYLQDQQLLGLWGCSGKLICTTAVPWNTSWSNKSQTDIWDNMTWMQWDKEIGNYTGEIYRLLEESQNQQEKNEKDLLALDSWKNLWNWFDITNWLWYIKIFIMIVGGLIGLRIIFAVLSIVNRVRQGYSPLSLQTLTQNPGGLDRLGRIEEEGGEQDKDRSIRLVNGFFALFWDDLRSLCLFSYHRLRDFILIVARAVELLGRSSLRGLQRGWEILKYLGSLLQYWGLELKKSAINLLDTIAIAVAEGTDRIIELIQRICRAICNIPRRIRQGFEAALQ

SEQ ID NO: 32 - protein, 716 aa, Artificial Sequence
  C1D7 sequence
MRVRGIQRNWPQWWIWGILGFWMIIICRVMGNLWVTVYYGVPVWKEAKTTLFCASDAKAYEKEVHNVWATHACVPTDPNPQEMVLENVTENFNMWKNDMVDQMHEDIIRLWDQSLKPCVKLTPLCVTLECRNVRNVSSNGTYNIIHNETYKEMKNCSFNATTVVEDRKQKVHALFYRLDIVPLDENNSSEKSSENSSEYYRLINCNTSAITQACPKVSFDPIPIHYCAPAGYAILKCNNKTFNGTGPCNNVSTVQCTHGIKPVVSTQLLLNGSLAEEEIIIRSENLTNNAKTIIVHLNETVNITCTRPNNNTRKSIRIGPGQTFYATGDIIGDIRQAHCNLSRDGWNKTLQGVKKKLAEHFPNKTINFTSSSGGDLEITTHSFNCRGEFFYCNTSGLFNGTYMPNGTNSNSSSNITLPCRIKQIINMWQEVGRAMYAPPIAGNITCRSNITGLLLTRDGGSNNGVPNDTETFRPGGGDMRNNWRSELYKYKVVEVKPLGVAPTEAKRRVVEREKRAVGIGAVFLGILGAAGSTMGAASITLTVQARQLLSGIVQQQSNLLRAIEAQQHMLQLTVWGIKQLQTRVLAIERYLQDQQLLGLWGCSGKLICTTAVPWNTSWSNKSQTDIWDNMTWMQWDKEIGNYTGEIYRLLEESQNQQEKNEKDLLALDSWKNLWNWFDITNWLWYIKIFIMIVGGLIGLRIIFAVLSIVNRVRQGY

SEQ ID NO: 33 - DNA, 2127 bp, Artificial Sequence
  nucleotide sequence encoding sC1
atgagagtgcggggcattcagagaaactggccccagtggtggatctggggcatcctgggcttttggatgatcattatctgccgcgtgatgggcaacctgtgggtcaccgtgtactacggcgtgcccgtgtggaaagaggccaagaccaccctgttctgcgccagcgacgccaaggcctacgagaaagaggtgcacaacgtctgggccacccacgcctgtgtgcccaccgaccccaatccccaggaaatggtcctggaaaacgtgaccgagaacttcaacatgtggaagaacgacatggtggaccagatgcacgaggacatcatccggctgtgggaccagagcctgaagccctgcgtgaagctgacccctctgtgcgtgaccctggaatgccggaacgtgcgcaacgtgtccagcaacggcacctacaatatcatccacaacgagacatacaaagagatgaagaactgcagcttcaacgctaccaccgtggtcgaggaccggaagcagaaggtgcacgccctgttttaccggctggacatcgtgcccctggacgagaacaacagcagcgagaagtcctccgagaacagctccgagtactacagactgatcaactgcaacaccagcgccatcacccaggcctgccccaaggtgtccttcgaccctatccccatccactactgcgcccctgccggctacgccatcctgaagtgcaacaacaagaccttcaatggcaccggcccctgcaacaatgtgtccaccgtgcagtgcacccacggcatcaagcccgtggtgtctacccagctgctgctgaacggcagcctggccgaggaagagatcatcatcagaagcgagaacctgaccaacaacgccaagacaatcatcgtccacctgaacgaaaccgtgaacatcacctgtacccggcctaacaacaacacccggaagtccatccggatcggccctggccagaccttttacgccaccggcgatattatcggcgacatccggcaggcccactgcaatctgagccgggacggctggaacaagacactgcagggcgtcaagaagaagctggccgaacacttccccaacaaaaccatcaacttcaccagctcctctggcggcgacctggaaatcaccacccacagctttaactgcagaggcgagttcttctactgcaatacctccggcctgttcaatggaacctacatgcccaacgggaccaacagcaactccagcagcaatatcaccctgccttgccggatcaagcagattatcaatatgtggcaggaagtgggcagagctatgtacgcccctccaatcgccggcaacatcacatgcagaagcaacattaccggcctgctgctcaccagggacggcggctctaacaatggcgtgccaaacgacaccgagacattcagacccggcggaggcgacatgcggaacaattggcggagcgagctgtacaagtacaaggtggtggaagtgaagcccctgggcgtggcccctaccgaagccaagagaagagtggtcgaacgcgaggaacgggccgtgggcattggagccgtgtttctgggaatcctgggagccgctggcagcaccatgggcgctgcctctatcacactgacagtgcaggccagacagctcctgagcggcatcgtgcagcagcagagcaacctgctgagagccatcgaggcacagcagcacatgctgcagctgaccgtgtggggcattaagcagctccagacacgggtgctggccattgagagatacctgcaggatcagcagctgctcggcctgtggggctgtagcggcaagctgatctgtaccaccgccgtgccttggaacacctcctggtccaacaagagccagaccgacatctgggacaacatgacctggatgcagtgggacaaagaaatcggcaactataccggcgagatctaccgactgctggaagagtcccagaaccagcaggaaaagatgaagcagatcgaggacaagatcgaagagattctgagcaaaatctaccacatcgagaacgagatcgcccgcatcaagaaactgatcggcgaagtgggatccggcgctcccacaaaggccaaaagacgggtggtgcagcgcgagaaacgc

SEQ ID NO: 34 - DNA, 2601 bp, Artificial Sequence
  nucleotide sequence encoding C1
atgagagtgcggggcattcagagaaactggccccagtggtggatctggggcatcctgggcttttggatgatcattatctgccgcgtgatgggcaacctgtgggtcaccgtgtactacggcgtgcccgtgtggaaagaggccaagaccaccctgttctgcgccagcgacgccaaggcctacgagaaagaggtgcacaacgtctgggccacccacgcctgtgtgcccaccgaccccaatccccaggaaatggtcctggaaaacgtgaccgagaacttcaacatgtggaagaacgacatggtggaccagatgcacgaggacatcatccggctgtgggaccagagcctgaagccctgcgtgaagctgacccctctgtgcgtgaccctggaatgccggaacgtgcgcaacgtgtccagcaacggcacctacaatatcatccacaacgagacatacaaagagatgaagaactgcagcttcaacgctaccaccgtggtcgaggaccggaagcagaaggtgcacgccctgttttaccggctggacatcgtgcccctggacgagaacaacagcagcgagaagtcctccgagaacagctccgagtactacagactgatcaactgcaacaccagcgccatcacccaggcctgccccaaggtgtccttcgaccctatccccatccactactgcgcccctgccggctacgccatcctgaagtgcaacaacaagaccttcaatggcaccggcccctgcaacaatgtgtccaccgtgcagtgcacccacggcatcaagcccgtggtgtctacccagctgctgctgaacggcagcctggccgaggaagagatcatcatcagaagcgagaacctgaccaacaacgccaagacaatcatcgtccacctgaacgaaaccgtgaacatcacctgtacccggcctaacaacaacacccggaagtccatccggatcggccctggccagaccttttacgccaccggcgatattatcggcgacatccggcaggcccactgcaatctgagccgggacggctggaacaagacactgcagggcgtcaagaagaagctggccgaacacttccccaacaaaaccatcaacttcaccagctcctctggcggcgacctggaaatcaccacccacagctttaactgcagaggcgagttcttctactgcaatacctccggcctgttcaatggaacctacatgcccaacgggaccaacagcaactccagcagcaatatcaccctgccttgccggatcaagcagattatcaatatgtggcaggaagtgggcagagctatgtacgcccctccaatcgccggcaacatcacatgcagaagcaacattaccggcctgctgctcaccagggacggcggctctaacaatggcgtgccaaacgacaccgagacattcagacccggcggaggcgacatgcggaacaattggcggagcgagctgtacaagtacaaggtggtggaagtgaagcccctgggcgtggcccctaccgaagccaagagaagagtggtcgaacgcgagaagcgggccgtgggcattggagccgtgtttctgggaatcctgggagccgctggcagcaccatgggcgctgcctctatcacactgacagtgcaggccagacagctcctgagcggcatcgtgcagcagcagagcaacctgctgagagccatcgaggcacagcagcacatgctgcagctgaccgtgtggggcattaagcagctccagacacgggtgctggccattgagagatacctgcaggatcagcagctgctcggcctgtggggctgtagcggcaagctgatctgtaccaccgccgtgccttggaacacctcctggtccaacaagagccagaccgacatctgggacaacatgacctggatgcagtgggacaaagaaatcggcaactataccggcgagatctaccgactgctggaagagtcccagaaccagcaggaaaagaacgagaaggacctgctggccctggacagctggaaaaatctgtggaattggttcgacatcaccaactggctgtggtacatcaagatcttcatcatgatcgtgggcggcctgatcggcctgcggatcatctttgccgtgctgagcatcgtgaaccgcgtgcggcagggatacagccctctgagcctgcagaccctgacccagaatccaggcggactggatcggctgggccggattgaggaagaaggcggcgagcaggacaaggaccgcagcatcagactcgtgaacggcttcttcgctctgttttgggacgacctgcggagcctgtgcctgttctcctaccacagactgcgggactttatcctgattgtggccagagccgtcgagctgctgggcagatcttctctgagaggcctgcagcggggctgggagattctgaagtacctgggctccctgctgcagtattggggcctggaactgaagaagtccgccatcaatctgctcgacacaatcgctattgccgtggccgaaggcaccgacagaatcatcgagctgatccagcggatctgccgggccatctgcaacatccccagacggatcagacagggctttgaagccgccctccag

SEQ ID NO: 35 - DNA, 2148 bp, Artificial Sequence
  nucleotide sequence encoding C1D7
atgagagtgcggggcattcagagaaactggccccagtggtggatctggggcatcctgggcttttggatgatcattatctgccgcgtgatgggcaacctgtgggtcaccgtgtactacggcgtgcccgtgtggaaagaggccaagaccaccctgttctgcgccagcgacgccaaggcctacgagaaagaggtgcacaacgtctgggccacccacgcctgtgtgcccaccgaccccaatccccaggaaatggtcctggaaaacgtgaccgagaacttcaacatgtggaagaacgacatggtggaccagatgcacgaggacatcatccggctgtgggaccagagcctgaagccctgcgtgaagctgacccctctgtgcgtgaccctggaatgccggaacgtgcgcaacgtgtccagcaacggcacctacaatatcatccacaacgagacatacaaagagatgaagaactgcagcttcaacgctaccaccgtggtcgaggaccggaagcagaaggtgcacgccctgttttaccggctggacatcgtgcccctggacgagaacaacagcagcgagaagtcctccgagaacagctccgagtactacagactgatcaactgcaacaccagcgccatcacccaggcctgccccaaggtgtccttcgaccctatccccatccactactgcgcccctgccggctacgccatcctgaagtgcaacaacaagaccttcaatggcaccggcccctgcaacaatgtgtccaccgtgcagtgcacccacggcatcaagcccgtggtgtctacccagctgctgctgaacggcagcctggccgaggaagagatcatcatcagaagcgagaacctgaccaacaacgccaagacaatcatcgtccacctgaacgaaaccgtgaacatcacctgtacccggcctaacaacaacacccggaagtccatccggatcggccctggccagaccttttacgccaccggcgatattatcggcgacatccggcaggcccactgcaatctgagccgggacggctggaacaagacactgcagggcgtcaagaagaagctggccgaacacttccccaacaaaaccatcaacttcaccagctcctctggcggcgacctggaaatcaccacccacagctttaactgcagaggcgagttcttctactgcaatacctccggcctgttcaatggaacctacatgcccaacgggaccaacagcaactccagcagcaatatcaccctgccttgccggatcaagcagattatcaatatgtggcaggaagtgggcagagctatgtacgcccctccaatcgccggcaacatcacatgcagaagcaacattaccggcctgctgctcaccagggacggcggctctaacaatggcgtgccaaacgacaccgagacattcagacccggcggaggcgacatgcggaacaattggcggagcgagctgtacaagtacaaggtggtggaagtgaagcccctgggcgtggcccctaccgaagccaagagaagagtggtcgaacgcgagaagcgggccgtgggcattggagccgtgtttctgggaatcctgggagccgctggcagcaccatgggcgctgcctctatcacactgacagtgcaggccagacagctcctgagcggcatcgtgcagcagcagagcaacctgctgagagccatcgaggcacagcagcacatgctgcagctgaccgtgtggggcattaagcagctccagacacgggtgctggccattgagagatacctgcaggatcagcagctgctcggcctgtggggctgtagcggcaagctgatctgtaccaccgccgtgccttggaacacctcctggtccaacaagagccagaccgacatctgggacaacatgacctggatgcagtgggacaaagaaatcggcaactataccggcgagatctaccgactgctggaagagtcccagaaccagcaggaaaagaacgagaaggacctgctggccctggacagctggaaaaatctgtggaattggttcgacatcaccaactggctgtggtacatcaagatcttcatcatgatcgtgggcggcctgatcggcctgcggatcatctttgccgtgctgagcatcgtgaaccgcgtgcggcagggctac

SEQ ID NO: 36 - protein, 724 aa, Artificial Sequence
  mosaic Env trimer sequence
MRVRGIQRNCQHLWRWGTLILGMLMICSAAGKLWVTVYYGVPVWKEATTTLFCASDAKAYDTEVHNVWATHACVPTDPNPQEVVLENVTENFNMWKNNMVEQMHEDIISLWDQSLKPCVKLTPLCVTLNCTDDVRNVTNNATNTNSSWGEPMEKGEIKNCSFNITTSIRNKVQKQYALFYKLDVVPIDNDSNNTNYRLISCNTSVITQACPKVSFEPIPIHYCAPAGFAILKCNDKKFNGTGPCTNVSTVQCTHGIRPVVSTQLLLNGSLAEEEVVIRSENFTNNAKTIMVQLNVSVEINCTRPNNNTRKSIHIGPGRAFYTAGDIIGDIRQAHCNISRANWNNTLRQIVEKLGKQFGNNKTIVFNHSSGGDPEIVMHSFNCGGEFFYCNSTKLFNSTWTWNNSTWNNTKRSNDTEEHITLPCRIKQIINMWQEVGKAMYAPPIRGQIRCSSNITGLLLTRDGGNDTSGTEIFRPGGGDMRDNWRSELYKYKVVKIEPLGVAPTKAKERVVQREERAVGIGAVFLGFLGAAGSTMGAASMTLTVQARLLLSGIVQQQNNLLRAIEAQQHLLQLTVWGIKQLQARVLAVERYLKDQQLLGIWGCSGKLICTTTVPWNASWSNKSLDKIWNNMTWMEWEREINNYTSLIYTLIEESQNQQEKNEQELLELDKWASLWNWFDISNWLWYIKSRIEGRGSGGYIPEAPRDGQAYVRKDGEWVLLSTFL

SEQ ID NO: 37 - protein, 28 aa, Artificial Sequence
  Residues 655-682 of SEQ ID NO:18
NEKDLLALDSWNNLWNWFSISKWLWYIK

SEQ ID NO: 38 - DNA, 4056 bp, Artificial Sequence
  nucleotide sequence of Mos1Gag-Pol antigen
atgggagctagagccagtgtgctgagcggcggagagctggatagatgggagaaaattcggctgcggccaggcggcaaaaagaagtatcgcctgaaacatattgtgtgggcctctcgcgagctggaaagatttgctgtgaatcctggactgctcgagacatctgaaggctgccgccagatcctcggtcaactgcagccatctctgcagaccggctcagaagagctgagatctctgtataatactgtcgccacactctattgcgtccaccagcgcattgaaatcaaagatacaaaggaggctctggagaagatagaagaggaacagaataagtctaaaaagaaggctcagcaggccgctgccgataccggcaacagctctcaggtctcacaaaattaccctatcgttcagaatattcaaggtcaaatggtccatcaggctatcagccctcgcacactgaatgcttgggtgaaagtggtcgaggaaaaagcctttagtccagaggttatacctatgtttagcgcactgtctgaaggagccactcctcaggacctcaataccatgctgaatactgtcggaggccatcaggccgctatgcaaatgctgaaagaaaccattaacgaggaagccgccgaatgggatcgagtgcatccagtccatgcaggaccaatcgctccaggccagatgagagaacctcgaggctctgatatcgccggaaccacaagcacactgcaggaacagattggatggatgacaaacaatcctcctatccctgtcggcgagatctataagagatggattatcctcggcctcaacaagattgtcagaatgtattcacctgtgtccattctggatatccgccaaggacctaaagagccattccgcgattacgtcgaccgcttttacaaaaccctgagagctgagcaggcatctcaggatgtcaaaaattggatgacagaaactctcctggtccagaacgctaatcctgattgcaagacaattctgaaggctctgggaccagccgccactctcgaggaaatgatgaccgcttgtcagggagtcggaggacctggacacaaggcaagagtgctcgctgaagccatgtctcaggtcacaaacagcgccacaattatgatgcagcgcggtaacttcagaaaccagcggaaaaccgtcaagtgttttaattgcggtaaagagggccatattgccaaaaattgcagagctcctcggaaaaagggctgctggaaatgtggaaaagaaggtcatcaaatgaaggattgcacagaacgccaggccaatttccttgggaagatttggccttccaacaaaggccgaccaggaaactttctgcagaatcggcctgagcctaccgctccacctgaagagagctttagattcggcgaggaaacaaccacaccatctcagaaacaagagcctattgataaggaaatgtatcctctggcttctctgaagtctctgttcggcaatgatcctagctcacaaatggctcccattagtcctattgaaacagtgcctgtgaaactgaaacctggaatggacggtcctagagtcaagcagtggcctctcacagaagagaagattaaggcactcaccgctatttgcgaagagatggagaaagaaggcaagattacaaagattggacctgagaatccatacaatacacctgtctttgccatcaaaaagaaagattctaccaaatggcgcaagctcgtggatttcagagaactcaacaaacgcacacaggatttttgggaggtccagctcggaattcctcatccagccggactgaaaaagaagaagtccgtcacagtcctggcagtcggcgacgcctatttctccgtgcctctcgatgaaggttttaggaagtataccgcctttacaattccatccacaaacaacgaaacaccaggcatccggtaccagtataatgtcctgccacaaggatggaagggatctcctgccatctttcagtgttccatgacacggatccttgaacctttcagagccaagaatccagagattgtgatctatcaatacatggccgcactctatgtcggatctgacctcgagattggacagcaccgcgccaagatcgaagagctgagagaacatctgctgaaatggggctttacaacaccagataagaaacatcagaaagaacctccttttctttggatgggatatgaactgcatcccgacaaatggacagtccagcctatccagctgccagagaaggatagctggaccgttaatgatattcagaagctcgttggtaaactgaattgggccagtcaaatctatcctggaatcaaagtccgacagctgtgcaagctgctcagaggcgccaaggctctcaccgatattgtgcctctgaccgaagaggctgaactggagctggccgagaatagagaaatcctcaaggagcctgtccacggcgtctactacgatccttctaaagacctgatcgctgaaatccaaaagcaaggacatgatcaatggacatatcagatctaccaggagccttttaagaatcttaagaccggcaagtatgccaaaatgcgcaccgctcatacaaatgacgtgaaacagctcaccgaggctgtccagaaaattgctatggaatctatcgtcatttggggcaaaacacctaaattccggcttcctattcagaaagaaacctgggagacatggtggacagattactggcaagctacatggatccctgaatgggaatttgtgaatacacctcctctcgtcaaactgtggtaccagttggagaaggatccaatcgccggcgtggaaacattctatgtggcaggcgccgctaacagagaaactaagctcggcaaggccggatatgtgacagacagaggtagacagaagattgtatctctgacagagacaacaaatcagaaaaccgctctccaggctatctacctcgcactgcaggattccggcagcgaagtgaatattgtgaccgcctctcagtatgcactcggaattattcaggcacagcctgataagtccgagtccgagctggtcaatcagatcatcgaacagctgattaagaaggaaagagtctacctgtcttgggtgccagcacacaagggaatcggcggcaatgaacaggtggacaaacttgtgtcctccggtattagaaaggtcctgttcctcgatggaattgacaaggctcaggaagaacacgagaaatatcactccaactggagagctatggcctccgatttcaatctgccacctgttgtggctaaggaaattgtcgcttcctgcgatcagtgtcaactcaaaggcgaagctatgcatggacaggtcgactgttctcctggaatatggcaactcgcttgtacacacctcgaaggcaaaatcatcctcgtggctgtccatgtggcctccggctatattgaagccgaagtgattcctgctgaaaccggccaggaaaccgcttactttattctgaaactcgctggacggtggcctgtgaaagtgattcataccgccaatggctccaacttcaccagcgccgctgtgaaagccgcttgctggtgggccggaatccagcaggagttcggaataccgtataaccctcagtcacaaggagtggtcgcctctatgaacaaggaattgaagaaaatcataggtcaagtccgagaccaagccgaacacctcaagaccgctgtccagatggcagtctttatccacaatttcaagcgcaaaggcggcattggcggctacagtgccggcgagagaattatcgacataatcgccacagacattcagacaaaggagctccagaagcagataatcaagatacagaatttccgcgtgtactaccgcgactctagagaccctatatggaagggtccagctaagctcttgtggaagggcgaaggcgctgtggtcattcaggacaattccgatatcaaggtcgttcctcggcggaaagtcaagatcattaaggattatggtaaacaaatggccggagctgattgcgtggcaggccggcaggacgaagattgataa

SEQ ID NO: 39 - DNA, 2061 bp, Artificial Sequence
  nucleotide sequence of Mos1Env antigen
atgcgcgtgaccggcatcaggaaaaactatcagcatctgtggagatggggtacaatgctcctcggaattctcatgatctgtagcgccgctggcaaactgtgggttacagtctattatggcgttccagtgtggaaagaagctacaacaacactgttctgtgcctccgatgccaaggcctatgatacagaagtgcataacgtctgggctacacatgcttgtgtgcctaccgatcctaatcctcaggaggtcgtcctcgaaaacgtcacagaaaactttaatatgtggaaaaacaatatggtcgaacagatgcacgaagatatcatttctctgtgggatcagagtctcaagccttgtgtgaaactgacacctctgtgcgtcacactcaattgcacagatgatgtccggaacgtcacaaacaatgctacaaataccaactcctcctggggtgaacctatggaaaaaggcgaaatcaaaaattgttcctttaatatcacaaccagcatccgcaacaaagtccagaaacagtatgctctcttttacaaactcgacgtcgtgcctatcgataatgactccaacaatacaaattaccgcctcatctcctgtaacacctccgtgattactcaggcctgtcctaaagtctcttttgagcctatcccaattcactattgtgcacctgctggatttgccatcctcaagtgtaatgacaagaagtttaacggtaccggtccttgtaccaacgtgtccacagtgcagtgtacacacggaattagacctgtggtgtctactcagctgctcctgaatggctctctggccgaagaggaagtcgtgattcggagcgagaactttacaaataacgctaaaacaatcatggtccagctcaatgtctccgtcgagattaactgtaccagacctaacaataacactcgcaagtccatccacattggaccaggacgcgccttttacaccgctggtgacattatcggagatatcaggcaggcacactgtaatatctctcgcgccaactggaacaacactctcagacagattgtcgagaagctcggtaaacagtttggtaacaacaaaacaatcgtctttaatcacagctctggcggcgatcctgagatcgtcatgcattccttcaattgcggaggggagttcttttattgcaactctaccaagctctttaactccacatggacttggaataacagcacatggaacaataccaaacgctccaacgatacagaggaacacatcactttgccatgcagaatcaagcaaatcattaacatgtggcaagaggtgggtaaagccatgtatgctcctcctatcagaggacagatcagatgcagctccaacattacaggcctgctcctgacaagagatggcggaaacgacacctccggaacagagatcttcagaccaggcggaggagacatgagagacaactggagaagcgaactctataagtataaggtcgtcaagattgagccacttggagtggctcccacaaaggccaagagacgcgtggtgcagtccgaaaagtccgccgtcggaattggagctgtgtttctcggatttctgggagctgccggctctaccatgggagcagcctccatgacactgacagtccaggctagactgctgctgagtggcattgtccagcaacagaacaatctcctgagagccattgaagctcagcaacatctcctccagctcacagtctggggcatcaaacagctccaggcaagagtgctcgccgtcgagcggtacctgaaagaccagcaactcctcggcatttggggctgttccggaaaactgatctgcaccacaacagttccctggaatgcctcttggagcaacaaatctctcgataagatttggaataacatgacttggatggagtgggaaagagaaatcaacaactacacctctctcatctacacactcatcgaagagtctcaaaatcagcaagaaaagaatgaacaggagctcctcgagctggataagtgggcttctctctggaattggttcgatatctctaactggctctggtgataa

SEQ ID NO: 40 - DNA, 4029 bp, Artificial Sequence
  nucleotide sequence of Mos2 Gag-Pol antigen
atgggcgccagagcctctatcctgcgcggaggcaaactggataagtgggaaaagattagactccgacctggcggtaaaaagcattatatgctcaaacacctcgtctgggctagcagagaactcgagagattcgctctgaaccctggtctcctggaaacatccgaagggtgtaaacagattatcaaacagctccagcctgcactccagactggaacagaggaacttcgctctctgtttaataccgtggctacactgtattgtgtgcacgctgaaatcgaagtccgcgacacaaaagaagctctcgacaaaattgaggaagagcagaacaaatctcagcagaagacacagcaggctaaggaagccgacggaaaagtgagccagaattatcccattgtccaaaatctccaaggacagatggtgcatcagccaatctctccaagaacactcaacgcctgggtcaaggtcatagaagagaaggcattctcacctgaagtcattccaatgttcaccgctctgtccgaaggcgcaacaccacaggatctgaacactatgctcaataccgtcggcggacaccaggcagcaatgcagatgctcaaggatacaatcaatgaagaggcagctgagtgggatagactccatcctgtgcatgccggtccagtcgcacctggacagatgcgcgagcctagaggctccgacattgctggcacaaccagtaacctccaggagcagatcgcttggatgacttccaatccacctattccagtcggagatatctacaaacgctggatcattctcggtctgaacaaaatcgtgcggatgtactctcctaccagcatcctcgatattaagcaaggtccaaaagaaccttttcgagactatgtcgacagattctttaaaacactgcgcgcagaacaggctacacaggacgtgaagaactggatgactgatacactcctcgtgcagaatgcaaatccagactgtaaaacaatcctgagagctctcggtccaggcgctacactggaagagatgatgactgcatgtcaaggtgtcggtggacctagccacaaagctcgcgtgctggcagaggctatgtcacagaccaattccacaatcctcatgcaacgctccaatttcaaaggctccaagcgcattgtcaaatgctttaactgtggcaaagaaggacatatcgctcggaattgccgcgcaccacgcaagaaaggatgttggaagtgcggcaaggaaggacatcagatgaaagactgtactgagagacaagctaattttctcggcaaaatctggccatctcacaaaggacgacctggaaatttcctgcagtctcggccagaacctacagctcctcctgccgagtccttcagattcgaagagactacaccagctcctaaacaggaacctaaggatagagaacctctgacctctctgcgcagcctgtttggctccgatcctctgtcccagatggcaccaatttctccaatcgaaaccgttcctgtcaagctcaagccaggcatggatggaccaaaagtcaaacaatggccactcactgaggagaaaatcaaggctctggtcgaaatctgcacagaaatggaaaaggaaggaaagatttccaaaatcggaccagaaaatccttacaacacacctatctttgctattaagaagaaggactccacaaagtggcgaaagctggtcgactttcgcgagctgaacaagagaactcaggacttctgggaagtgcaactcggtattccacatcctgcaggactcaagaaaaagaaatctgtcactgtgctcgccgtcggtgacgcttacttttctgtgccactggatgaagattttcgcaagtacaccgcattcacaatcccttccattaacaatgagacacctggtattcgctatcagtacaatgtgcttcctcaaggctggaaaggtagtcctgctattttccagtcctctatgacaaagattcttgagccttttcgcaaacagaatcctgatatcgtcatctaccagtatatggcagctctgtacgtcggctctgatctggaaatcggccagcatagaactaagattgaggaactccgacagcacctgctccgctggggttttactactcctgacaagaagcaccagaaggaaccaccattcctctggatgggttacgaacttcatcctgataagtggactgtgcagccaattgtcctgcctgaaaaggattcttggacagtcaatgacatccagaaactcgtcggaaaactcaactgggcttctcagatctatgccggcattaaggtcaagcagctctgcaaactcctgagaggcacaaaggcactgacagaagtggttcctctcactgaagaagcagaactcgaactcgctgagaaccgcgaaattctcaaagaaccagtgcatggtgtctattatgatccaagcaaagatctcattgcagagattcagaaacaaggccaaggccagtggacttaccaaatctatcaggaacctttcaaaaatctcaagacaggcaaatacgctcggatgcgaggcgctcacaccaatgatgtcaagcaactcacagaggcagtgcagaagattgccacagagtctattgtgatctggggaaagactccaaagtttaagcttccaatccaaaaggagacttgggaagcttggtggactgaatattggcaggcaacttggattccagagtgggagtttgtcaatactccaccactcgtgaagctctggtatcagctcgagaaagagcctatcgtcggcgccgaaaccttttatgtcgctggtgccgcaaaccgcgagacaaaactcggaaaagcaggatacgtcaccgatagaggacggcagaaggtcgtcagcctgaccgacactactaaccagaagactgcacttcaggcaattcatctggctctccaggatagcggtctggaagtcaatatcgtcaccgctagtcagtacgctctgggtattatccaggctcagccagacaaaagcgaatccgaactcgtgtctcagattattgagcagctcatcaagaaagagaaagtctatctcgcctgggttccggctcacaaaggcattggtggaaatgagcaagtcgataagctcgtcagcagaggaatcaggaaagtcctcttcctggacggtatcgataaggcacaggaggaacatgagaagtaccacagtaactggcgcgccatggcttctgagtttaacctgcctccaatcgtcgccaaagagatcgtggcaagctgtgacaaatgtcagctgaaaggagaggcaatccatggccaggttgactgctcaccaggaatttggcagctcgcctgcactcatctggaaggaaaagtgattctggtcgctgtgcatgtcgctagtggctacatcgaggctgaggtcatacctgcagagacaggacaggagactgcttattttctgctcaagctcgccggaagatggccagtcaagaccattcacaccgctaacggctctaatttcacaagcgccacagtcaaagcagcatgttggtgggctggtatcaaacaggaattcggcattccttataatccacagtctcaaggcgtcgtggctagtatcaacaaagaactcaaaaagatcattggccaagtcagagaccaggctgagcatctcaaaactgcagtgcaaatggctgtgtttattcataactttaagagaaaaggtggcatcggcgagtacagcgctggcgagcgcatcgtggatattattgcttcagatatacagactaaggaactgcagaaacaaattaccaagatccagaactttagagtctactacagagattctcgagatcctctctggaaaggaccagcaaaacttctgtggaaaggagaaggtgcagtcgtgatccaggataactctgacatcaaagtggtgcctcggagaaaggccaaaatcattagagattacggaaagcagatggcaggcgatgattgtgtcgctagtagacaggatgaggattgataa

SEQ ID NO: 41 - DNA, 2139 bp, Artificial Sequence
  nucleotide sequence of Env Mos2-C4D7 antigen
atgcgagtcagaggtatgctgagaaattggcagcagtggtggatttggtccagcctcggattctggatgctgatgatctacagcgtcatgggtaatctctgggtcacagtgtattacggagttcctgtctggaaggacgccaagactacactcttttgcgcctctgacgccaaagcttacgaaaaggaagtccacaatgtgtgggcaactcatgcctgtgttcctacagatccaaatccacaggagatcgtgctcggcaatgtcaccgagaatttcaacatgtggaagaatgatatggtggatcaaatgcatgaggacatcatttccctctgggacgcctctctggaaccatgtgtcaagctcactccactgtgtgtgaccctcaactgcagaaacgtgcgcaacgtgtcctccaatggcacatacaatatcattcataatgagacttataaggaaatgaagaattgctctttcaatgccaccacagtcgtcgaggatcgcaaacagaaagtccatgctctgttttaccggctggatatcgttcctctcgatgagaacaattcctccgagaagtcctctgagaactctagcgagtactacaggctcattaattgtaatacctctgccatcacacaggcttgtccaaaggtctccttcgatcctattcctatccattactgtgctcctgccggatacgctattctcaaatgtaacaacaagacattcaatggtactggtccatgcaacaatgtgtctaccgtccagtgcactcatggtattaagcctgtcgtcagtacacagctcctgctcaatggatctctcgctgaggaagaaatcattatcagaagtgaaaacctcactaacaacgccaaaaccattattgtccatctgaacgagacagtcaatatcacatgcacacgacctaataacaataccagaaagtctatcagaatcggacctggccagacattctatgccacaggcgatatcattggtgacattagacaggctcattgcaatctgtccagagatggttggaataagacactccaaggtgtcaagaagaaactcgccgaacactttcctaacaagaccattaagtttgcccctcactcaggcggtgacctcgagattacaacacacacctttaactgtagaggcgaattcttctactgtaacacaagcaacctcttcaacgagagcaacatcgagcggaacgacagcatcattacacttccatgtcgcatcaagcagatcattaatatgtggcaggaagtcggacgcgctatctacgctccacctattgccggaaacatcacatgtcggagcaatattaccggactcctgctcacacgcgacggtggctctaacaatggcgtgccaaatgataccgaaacctttagacctggtggaggcgacatgcgcaacaattggcgctctgaactgtacaagtacaaagtcgtcgaagtcaaacctctcggagtcgctcctaccgaggctaaacgcagagtggtggaacgcgagaagcgggctgtcggtatcggtgcagtgttcctaggcatcctcggcgcagccggcagcacaatgggcgctgcttctattacactcactgtgcaggccagacagctcctgagcggaattgtgcagcagcaatcaaatctgctgcgcgctatcgaagcacagcagcatatgctccaactgactgtttggggtattaagcaactgcagactagagtcctggccattgaacggtatctccaggatcagcagctgctcggactctggggatgctctggcaagctcatctgtacaacagctgtgccttggaacacttcctggtctaacaagtctcagaccgatatttgggataatatgacatggatgcagtgggataaggaaatcggtaattatacaggcgagatctaccgactgctcgaggaatctcagaatcaacaggagaagaacgaaaaggatctcctggctctcgactcctggaacaatctgtggaactggtttagcatttccaagtggctgtggtacatcaagatcttcatcatgatcgtgggcggcctgatcggcctgcggatcatctttgccgtgctgagcatcgtgaaccgcgtgcggcagggctactgataa

SEQ ID NO: 42 - DNA, 124 bp, Artificial Sequence
  Pr13.5 Long Promoter Sequence
taaaaatagaaactataatcatataatagtgtaggttggtagtattgctcttgtgactagagactttagttaaggtactgtaaaaatagaaactataatcatataatagtgtaggttggtagta

SEQ ID NO: 43 - DNA, 227 bp, Artificial Sequence
  PrHyb Promoter Sequence
gttttgaaaatttttttataataaatatccggtaaaaattgaaaaactattctaatttattgcacggtccggtaaaaattgaaaaactattctaatttattgcacggtccggtaaaaattgaaaaactattctaatttattgcacggtccggtaaaaattgaaaaactattctaatttattgcacggtccggtaaaaattgaaaaactattctaatttattgcacgg

SEQ ID NO: 44 - protein, 15 aa, Artificial Sequence
  Env peptide
IHIGPGRAFYTAGDI

SEQ ID NO: 45 - protein, 9 aa, Artificial Sequence
  Gag peptide
AMQMLKETI

SEQ ID NO: 46 - protein, 9 aa, Artificial Sequence
  Pol peptide
YYDPSKDLI